European Patent Specification EP 3 341 404 B1, published April 3, 2024. Title: NOVEL INSULIN ANALOGS AND USE THEREOF. Applicant: HANMI PHARM. CO., LTD. The sequence listing filed with the application follows.

SEQUENCE LISTING (24 sequences)

SEQ ID NO: 1 - protein, 21 aa, Homo sapiens
GIVEQCCTSICSLYQLENYCN

SEQ ID NO: 2 - protein, 30 aa, Artificial Sequence
  Homo sapiens
FVNQHLCGSHLVEALYLVCGERGFFYTPKT

SEQ ID NO: 3 - protein, 21 aa, Artificial Sequence
  Insulin A-chain
  MISC_FEATURE (1): Xaa is alanine, glycine, glutamine, histidine, glutamic acid, or asparagine
  MISC_FEATURE (5): Xaa is alanine, glutamic acid, glutamine, histidine, or asparagine
  MISC_FEATURE (12): Xaa is alanine, serine, glutamine, glutamic acid, histidine, or asparagine
  MISC_FEATURE (14): Xaa is alanine, tyrosine, glutamic acid, histidine, lysine, aspartic acid, or asparagine
  MISC_FEATURE (16): Xaa is alanine, leucine, tyrosine, histidine, glutamic acid, or asparagine
  MISC_FEATURE (19): Xaa is alanine, tyrosine, serine, glutamic acid, histidine, or asparagine
  MISC_FEATURE (21): Xaa is asparagine, glycine, histidine, or alanine
XIVEXCCTSICXLXQXENXCX

SEQ ID NO: 4 - protein, 30 aa, Artificial Sequence
  Insulin B-chain
  MISC_FEATURE (16): Xaa is tyrosine, glutamic acid, or aspartic acid, or is absent
  MISC_FEATURE (25): Xaa is phenylalanine, or is absent
  MISC_FEATURE (27): Xaa is threonine, or is absent
  MISC_FEATURE (28): Xaa is proline, glutamic acid, or aspartic acid, or is absent
FVNQHLCGSHLVEALXLVCGERGFXYXXKT

SEQ ID NO: 5 - DNA, 37 bp, Artificial Sequence
  Primer
ccagcatctgctccctcgaacagctggagaactactg

SEQ ID NO: 6 - DNA, 37 bp, Artificial Sequence
  Primer
cagtagttctccagctgttcgagggagcagatgctgg

SEQ ID NO: 7 - DNA, 34 bp, Artificial Sequence
  Primer
cagcatctgctccctcaaccagctggagaactac

SEQ ID NO: 8 - DNA, 34 bp, Artificial Sequence
  Primer
gtagttctccagctggttgagggagcagatgctg

SEQ ID NO: 9 - DNA, 34 bp, Artificial Sequence
  Primer
gcggggaacgaggcttctacacacccaagacccg

SEQ ID NO: 10 - DNA, 34 bp, Artificial Sequence
  Primer
cgggtcttgggtgtgtagaagcctcgttccccgc

SEQ ID NO: 11 - DNA, 34 bp, Artificial Sequence
  Primer
cagcatctgctccctcgcccagctggagaactac

SEQ ID NO: 12 - DNA, 34 bp, Artificial Sequence
  Primer
gtagttctccagctgggcgagggagcagatgctg

SEQ ID NO: 13 - DNA, 34 bp, Artificial Sequence
  Primer
ctggtggaagctctcgagctagtgtgcggggaac

SEQ ID NO: 14 - DNA, 34 bp, Artificial Sequence
  Primer
gttccccgcacactagctcgagagcttccaccag

SEQ ID NO: 15 - DNA, 261 bp, Artificial Sequence
  Insulin Analog 1
ttcgttaaccaacacttgtgtggctcacacctggtggaagctctctacctagtgtgcggggaacgaggcttcttctacacacccaagacccgccgggaggcagaggacctgcaggtggggcaggtggagctgggcgggggccctggtgcaggcagcctgcagcccttggccctggaggggtccctgcagaagcgtggcattgtggaacaatgctgtaccagcatctgctccctcgaacagctggagaactactgcaactga

SEQ ID NO: 16 - protein, 86 aa, Artificial Sequence
  Insulin Analog 1
FVNQHLCGSHLVEALYLVCGERGFFYTPKTRREAEDLQVGQVELGGGPGAGSLQPLALEGSLQKRGIVEQCCTSICSLEQLENYCN

SEQ ID NO: 17 - DNA, 261 bp, Artificial Sequence
  Insulin Analog 2
ttcgttaaccaacacttgtgtggctcacacctggtggaagctctctacctagtgtgcggggaacgaggcttcttctacacacccaagacccgccgggaggcagaggacctgcaggtggggcaggtggagctgggcgggggccctggtgcaggcagcctgcagcccttggccctggaggggtccctgcagaagcgtggcattgtggaacaatgctgtaccagcatctgctccctcaaccagctggagaactactgcaactga

SEQ ID NO: 18 - protein, 86 aa, Artificial Sequence
  Insulin Analog 2
FVNQHLCGSHLVEALYLVCGERGFFYTPKTRREAEDLQVGQVELGGGPGAGSLQPLALEGSLQKRGIVEQCCTSICSLNQLENYCN

SEQ ID NO: 19 - DNA, 258 bp, Artificial Sequence
  Insulin Analog 3
ttcgttaaccaacacttgtgtggctcacacctggtggaagctctctacctagtgtgcggggaacgaggcttctacacacccaagacccgccgggaggcagaggacctgcaggtggggcaggtggagctgggcgggggccctggtgcaggcagcctgcagcccttggccctggaggggtccctgcagaagcgtggcattgtggaacaatgctgtaccagcatctgctccctcgaacagctggagaactactgcaactga

SEQ ID NO: 20 - protein, 85 aa, Artificial Sequence
  Insulin Analog 3
FVNQHLCGSHLVEALYLVCGERGFYTPKTRREAEDLQVGQVELGGGPGAGSLQPLALEGSLQKRGIVEQCCTSICSLEQLENYCN

SEQ ID NO: 21 - DNA, 258 bp, Artificial Sequence
  Insulin Analog 4
ttcgttaaccaacacttgtgtggctcacacctggtggaagctctcgagctagtgtgcggggaacgaggcttctacacacccaagacccgccgggaggcagaggacctgcaggtggggcaggtggagctgggcgggggccctggtgcaggcagcctgcagcccttggccctggaggggtccctgcagaagcgtggcattgtggaacaatgctgtaccagcatctgctccctcgcccagctggagaactactgcaactga

SEQ ID NO: 22 - protein, 85 aa, Artificial Sequence
  Insulin Analog 4
FVNQHLCGSHLVEALELVCGERGFYTPKTRREAEDLQVGQVELGGGPGAGSLQPLALEGSLQKRGIVEQCCTSICSLAQLENYCN

SEQ ID NO: 23 - DNA, 30 bp, Artificial Sequence
  N-terminal fusion partner
atggcaacaacatcaacagcaactacgcgt

SEQ ID NO: 24 - protein, 10 aa, Artificial Sequence
  N-terminal fusion partner
MATTSTATTR